European Patent Application EP 4 775 216 A1, published July 15, 2026. Title: Central nervous system targeted pharmaceutical compositions. Applicant: China Medical University. Application EP. The sequence listing filed with the application follows.

SEQUENCE LISTING (5 sequences)

SEQ ID NO: 1 - protein, 116 aa, synthetic construct
QVQLQESGGGLVQAGGSLRLSCAASGRTFASNSMGWFRQAPGKEREFVAAINRGSGEIYYADSVKGRFTISRDNAKNTVYLQMNSLKPEDTAVYYCAAFRDLYDYWGQGTQVTVSS

SEQ ID NO: 2 - protein, 118 aa, synthetic construct
QVQLQESGGGLVQAGGSLRLSCAASGRTFASNSMGWFRQAPGKEREFVAAISRGSGSIYYADSVKGRFTISRDNAKNTVYLQMNSLKPEDTAVYYCAASRDLYRYDYWGQGTQVTVSS

SEQ ID NO: 3 - protein, 118 aa, synthetic construct
QVQLQESGGGLVQAGGSLRLSCAASGRTFSSNVMGWFRQAPGKEREFVAAINRGSGEIYYADSVKGRFTISRDNAKNTVYLQMNSLKPEDTAVYYCAASRDLYRYDYWGQGTQVTVSS

SEQ ID NO: 4 - protein, 118 aa, synthetic construct; identical to SEQ ID NO: 2

SEQ ID NO: 5 - protein, 118 aa, synthetic construct; identical to SEQ ID NO: 3